European Patent Specification EP 3 823 443 B1, published May 22, 2024. Title: Non-Human Animal Models of Ditra Disease and Uses Thereof. Applicant: Regeneron Pharmaceuticals, Inc. The sequence listing filed with the application follows.

SEQUENCE LISTING (57 sequences)

SEQ ID NO: 1 - DNA, 2628 bp, Homo sapiens
cccgcccacggtggcggggaaatacctaggcatggaagtggcatgacagggctcgtgtccctgtcatattttccactctccacgaggtcctgcgcgcttcaatcctgcaggcagcccggtttggggatgtggtccttgctgctctgcgggttgtccatcgcccttccactgtctgtcacagcagatggatgcaaggacatttttatgaaaaatgagatactttcagcaagccagccttttgcttttaattgtacattccctcccataacatctggggaagtcagtgtaacatggtataaaaattctagcaaaatcccagtgtccaaaatcatacagtctagaattcaccaggacgagacttggattttgtttctccccatggaatggggggactcaggagtctaccaatgtgttataaagggtagagacagctgtcatagaatacatgtaaacctaactgtttttgaaaaacattggtgtgacacttccataggtggtttaccaaatttatcagatgagtacaagcaaatattacatcttggaaaagatgatagtctcacatgtcatctgcacttcccgaagagttgtgttttgggtccaataaagtggtataaggactgtaacgagattaaaggggagcggttcactgttttggaaaccaggcttttggtgagcaatgtctcggcagaggacagagggaactacgcgtgtcaagccatactgacacactcagggaagcagtacgaggttttaaatggcatcactgtgagcattacagaaagagctggatatggaggaagtgtccctaaaatcatttatccaaaaaatcattcaattgaagtacagcttggtaccactctgattgtggactgcaatgtaacagacaccaaggataatacaaatctacgatgctggagagtcaataacactttggtggatgattactatgatgaatccaaacgaatcagagaaggggtggaaacccatgtctcttttcgggaacataatttgtacacagtaaacatcaccttcttggaagtgaaaatggaagattatggccttcctttcatgtgccacgctggagtgtccacagcatacattatattacagctcccagctccggattttcgagcttacttgataggagggcttatcgccttggtggctgtggctgtgtctgttgtgtacatatacaacatttttaagatcgacattgttctttggtatcgaagtgccttccattctacagagaccatagtagatgggaagctgtatgacgcctatgtcttataccccaagccccacaaggaaagccagaggcatgccgtggatgccctggtgttgaatatcctgcccgaggtgttggagagacaatgtggatataagttgtttatattcggcagagatgaattccctggacaagccgtggccaatgtcatcgatgaaaacgttaagctgtgcaggaggctgattgtcattgtggtccccgaatcgctgggctttggcctgttgaagaacctgtcagaagaacaaatcgcggtctacagtgccctgatccaggacgggatgaaggttattctcattgagctggagaaaatcgaggactacacagtcatgccagagtcaattcagtacatcaaacagaagcatggtgccatccggtggcatggggacttcacggagcagtcacagtgtatgaagaccaagttttggaagacagtgagataccacatgccgcccagaaggtgtcggccgtttcctccggtccagctgctgcagcacacaccttgctaccgcaccgcaggcccagaactaggctcaagaagaaagaagtgtactctcacgactggctaagacttgctggactgacacctatggctggaagatgacttgttttgctccatgtctcctcattcctacacctattttctgctgcaggatgaggctagggttagcattctagacacccagttgagctcaggcgtagagaagaggaggatgggataagaactggggccatccccatgtcatggtgggtgagagctggggccatccccgtggtcatggagggtgagagctgggggttatccccatggtcatggagggtgagggctggtcgggggaggcatccccaagtcatggtgggtgagagctcggagcatccccatgtcatggtgggtgagatctgggggtatccctgtgtcatggtgggtgagggcgggtggtcatccacatggtcatagtgggtgagagctgggggtatccctacatcatggtgggtgagagctgggagcatccccatgtcatggtgggcgagatctggggggtatccccacgtcatggtggatgagagctgggggaatcaccatgtcatggtgggtgagatcttgggggatcacctgtcatggtgggtgagagctggggggatcacctgtcatggtgggtgagagttgggattcatccccatgtcatggtgggctgagcccacatggaagcctgtgcttggacagcgtatgcccttttctctgtttttccacaatgaacaattaaactgtaaatgttaaaaatatcagtaatttgtgaaataaattttattctcatttgagcaacataaaaaaaaaaaaaaaa

SEQ ID NO: 2 - protein, 575 aa, Homo sapiens
MWSLLLCGLSIALPLSVTADGCKDIFMKNEILSASQPFAFNCTFPPITSGEVSVTWYKNSSKIPVSKIIQSRIHQDETWILFLPMEWGDSGVYQCVIKGRDSCHRIHVNLTVFEKHWCDTSIGGLPNLSDEYKQILHLGKDDSLTCHLHFPKSCVLGPIKWYKDCNEIKGERFTVLETRLLVSNVSAEDRGNYACQAILTHSGKQYEVLNGITVSITERAGYGGSVPKIIYPKNHSIEVQLGTTLIVDCNVTDTKDNTNLRCWRVNNTLVDDYYDESKRIREGVETHVSFREHNLYTVNITFLEVKMEDYGLPFMCHAGVSTAYIILQLPAPDFRAYLIGGLIALVAVAVSVVYIYNIFKIDIVLWYRSAFHSTETIVDGKLYDAYVLYPKPHKESQRHAVDALVLNILPEVLERQCGYKLFIFGRDEFPGQAVANVIDENVKLCRRLIVIVVPESLGFGLLKNLSEEQIAVYSALIQDGMKVILIELEKIEDYTVMPESIQYIKQKHGAIRWHGDFTEQSQCMKTKFWKTVRYHMPPRRCRPFPPVQLLQHTPCYRTAGPELGSRRKKCTLTTG

SEQ ID NO: 3 - DNA, 4072 bp, Mus musculus
ggcggacagagaccggaagctgggagatgatggcttctgatgtttgttgcttacgcgacacagcttgtttggaattatgtggcccttgacaactgcgtggcacacacttcaagatacaaaagtgagaagaagaggggggtcaccagaggagactgaagtcagtaagtttctaccaaagctgggtttcttctggccactccaaacaaagctgaaattgtccttcagacctctcctgagatgggggttacatctttgctcttctgtggggtgtttttcctgcttctgcttttcgtggcagcagatacgtgtgaggacatttttatgcacaatgtgataatttcagagggccagccttttcctttcaactgcacatacccgccagaaacaaacggggcagtaaatctgacatggtacaaaacacctagcaaaagcccagtatctaacaacagacaccttagagttcaccaggaccagacctggatcttgtttcttccattgacactggaggactccggtatctatcagtgtgttataaggaatgcccacaactgctaccaaatagctgtgaacctaaccgttttaaaaaaccactggtgtgactcttccatggaggggagtcccgtaaattcaccagatgtgtaccagcaaatattacccataggaaaatcgggcagtctgaattgtcatctctacttcccagaaagttgtgctttggattcaataaaatggtataagggttgtgaagagattaaagcggggaaaaagtacagcccttcaggagcaaagcttcttgtgaacaacgttgctgtggaggacggcgggagctatgcgtgctcagccagactgactcacttggggagacacttcaccattagaaactacattgctgtgaacaccaaggaagttgagtatggaagaaggatccctaacatcacgtatccaaagaacaactccattgaagttccacttggctccaccctcatcgtgaactgcaatataacagacacgaaggagaatacaaacctgaggtgctggagagtcaacaacaccctggtggatgactactacaaagactccaaacgcatccaggaaggaatcgaaaccaatgtgtccttgagggatcaaattcggtacacagtgaacataacattcttaaaagtgaaaatggaggactacggccgtcctttcacgtgtcatgctggagtgtccgcagcctacatcattctgatatacccagttccagacttcagggcttacctcttaggagggcttatggcgttcctacttctggttgtatctgttctgttcatctacaacagctttaagatcgacatcatgctttggtacagaagcgccttccacactgcccaggctccagatgatgagaagctgtatgatgcctatgtcttataccccaagtacccgagaggaagccagggccatgatgtagacacactggtactgaagatcttgcccgaggtgctggagaaacagtgtggatataagttatttatatttggcagggatgaattccctggacaagctgtggccagcgtcattgatgaaaacattaagctgtgtaggaggctgatggtctttgtggcaccagagtcgtctagcttcggctttctaaagaacttgtcagaagaacaaattgccgtctacaatgccctcatccagcatggcatgaaggtcattctgatcgaactggagaaagtcaaagactacagcaccatgcccgagtccattcagtatatccgacagaagcacggggccatccaatgggatggggacttcacagagcagtcacagtgtgccaagaccaagttctggaagaaagtgagataccatatgccacccaggaggtatccagcatcttccccagtccagctgctgggacacataccctgcaattgcaaggcaggcaaatgcaatgctgccacagggctcataactccctgagagtggttagtgtgtgttggctcacactacatcctctctgaattgtctactcatgtagctggctcttttgtgcttgtgagcgaccttgtccttgcccttgtagctttttgtttatttgtattgtttgctggatgctttcagtcatagctgatccttattactcctgtttgcttcatggctcctgaaaacccatatactccccaagcatggggtggctctaacgttgggcctccgtgtcagtgggatactgaggatgacagatcaggtgtccaggatgcttgatcctggtttgagatgggaggctgggcagtctgaggataccaagtagatagccttagggaagatcagcaaggacagtagtgcaatgtctgtgtttgtccagggtccacaagattctagtcctcaggcagtgtagactgcatttgaatctccttcattttcctattgcatttagttaactaaccattgtgagaacaggacagaggactgggagttgggggtggggggaggtgacagaggatgggagtgtgtgtgtaagaggtgacagttacatgatcaatcctgggaaatcagactcaggaaaccagcattagggtgcagatctgagttttttgtgcagcccttaagcttatatacagcgttcgagccaatcccaagcccctaaaccctcggccaatcatatcttgccacatcatcactatgcctcaatgaaagccctgcctgatgaggtaactcaaaaggaattggggtgggaagcatcatcccctgtcagaacttccgtgaagatggaggacgtagccactaccccacctcagtttctttttgttgtctcaggtttgcaccagagccatcttaaatctagtgacatgtgcagcaaatcatgactcttcaaggagctgcgggagcctgtggtgcctcgctctccatcccactttttccttcacagggttgacttccacgtcccccaaaccatggtattagcacgatgcccctagaagccgcttagatgtcgccaggaccaatggtcttcatttccctctttcccagcccctgtgaatcttactattctaggaaattcaaatgagagacacggtgcattcacggtttctcattttatgactggcttctttcatacaccacggatttctcaagtgctctcgagattcatccattgattagccttttgttttattattatcactactgtctttctcttctttttcttcctctttaaatttctccccctcctcacgagcatccggagaggagcatagactctctgcatgcctacagcgtgatgagctcaccgagggtcccttcaatcacaagcttgtatgttttgcttttcggtttctctttgcaccatgggaattgtaactccttacagaggatttgaaggttcgggtacaaaggcgtcactgactggttccttcttctgtcttcctcaccctgaatgggctttgcttctgggtgattcctggaaattgtcagcagtgatggagaaacctagggacagggctgactaatggggcctggcctttcttctttgaagcccaggacacagtgcctgcctagtgggtcctggacacaccaggtggttccactctgctcagtggtaacattttttagctgagtcatcaacatcgggtcctttagtgaggaggtgcgggcatctctccccagttagatttggactcttacttccctgctcatttccctttgaaagattcaggagactatgtcagaagcagggagccagcaccctgtgtcttctccacgtggctccttgtcacacctgtgaccaccaattttagaaaatgtgtttccttgttctgaccacacttatgcggacattagttgaggctgttgtcagaaaggaaaattaactcatttgaagtaaacattttctggaaatctctgacttctgtcaggccaatggtgctgaaaaatttaaaactgaattcacttttttggccagaaagctttcctcttgccaacatgtcttaattttccttttgcttaaacttattggagatgtattatgaatgctaagatgtgagtgtgttatatcagtacattgacattttaaataaagtatattttaataaaa

SEQ ID NO: 4 - protein, 574 aa, Mus musculus
MGVTSLLFCGVFFLLLLFVAADTCEDIFMHNVIISEGQPFPFNCTYPPETNGAVNLTWYKTPSKSPVSNNRHLRVHQDQTWILFLPLTLEDSGIYQCVIRNAHNCYQIAVNLTVLKNHWCDSSMEGSPVNSPDVYQQILPIGKSGSLNCHLYFPESCALDSIKWYKGCEEIKAGKKYSPSGAKLLVNNVAVEDGGSYACSARLTHLGRHFTIRNYIAVNTKEVEYGRRIPNITYPKNNSIEVPLGSTLIVNCNITDTKENTNLRCWRVNNTLVDDYYKDSKRIQEGIETNVSLRDQIRYTVNITFLKVKMEDYGRPFTCHAGVSAAYIILIYPVPDFRAYLLGGLMAFLLLVVSVLFIYNSFKIDIMLWYRSAFHTAQAPDDEKLYDAYVLYPKYPRGSQGHDVDTLVLKILPEVLEKQCGYKLFIFGRDEFPGQAVASVIDENIKLCRRLMVFVAPESSSFGFLKNLSEEQIAVYNALIQHGMKVILIELEKVKDYSTMPESIQYIRQKHGAIQWDGDFTEQSQCAKTKFWKKVRYHMPPRRYPASSPVQLLGHIPCNCKAGKCNAATGLITP

SEQ ID NO: 5 - DNA, 2044 bp, Rattus norvegicus
ccggctggcctaggatcaggcaagaaaaggctgaacgcctttctaaggacggactctttctgtacagctccacttggggaagcccgaaatggggatgccacccttgctcttctgttgggtgtctttcgtgcttccactttttgtggcagcaggtaactgtactgatgtctatatgcaccatgagatgatttcagagggccagcctttccccttcaactgcacataccctccagtaacaaacggggcagtgaatctgacatggcatagaacacccagtaagagcccaatctccatcaacagacacgttagaattcaccaggaccagtcctggattttgtttcttccgttggcattggaggactcaggcatctatcaatgtgttataaaggatgcccacagctgttaccgaatagctataaacctaaccgtttttagaaaacactggtgcgactcttccaacgaagagagttccataaattcctcagatgagtaccagcaatggttacccataggaaaatcgggcagtctgacgtgccatctctacttcccagagagctgtgttttggattcaataaagtggtataagggttgtgaagagattaaagtgagcaagaagttttgccctacaggaacaaagcttcttgttaacaacatcgacgtggaggatagtgggagctatgcatgctcagccagactgacacacttggggagaatcttcacggttagaaactacattgctgtgaataccaaggaagttgggtctggaggaaggatccctaacatcacgtatccaaaaaacaactccattgaagttcaacttggctccaccctcattgtggactgcaatataacagacacgaaggagaatacgaacctcagatgctggcgagttaacaacaccctggtggacgattactacaacgacttcaaacgcatccaggaaggaatcgaaaccaatctgtctctgaggaatcacattctgtacacagtgaacataacattcttagaagtgaaaatggaggactacggccatcctttcacatgccacgctgcggtgtccgcagcctacatcattctgaaacgcccagctccagacttccgggcttacctcataggaggtctcatggctttcctacttctggccgtgtccattctgtacatctacaacacctttaaggtcgacatcgtgctttggtataggagtaccttccacactgcccaggctccagatgacgagaagctgtatgatgcctatgtcttataccccaagtacccaagagaaagccagggccatgatgtggacacactggtgttgaagatcttgcccgaggtgctggagaaacagtgtggatataagttattcatatttggcagggatgaattccctggacaagctgtggccagcgtcattgatgaaaacattaagctgtgtaggaggctgatggtcctcgtggcaccagagacatccagcttcagctttctgaagaacttgactgaagaacaaatcgctgtctacaatgccctcgtccaggacggcatgaaggtcattctgattgaactggagagagtcaaggactacagcaccatgcccgagtccattcagtacatccgacagaagcacggggccatccagtgggatggggacttcacagagcaggcacagtgcgccaagacgaaattctggaagaaagtgagatatcatatgccacccaggaggtacccggcatctccccccgtccagctgctaggacacacaccccgcataccaggctagtgcagtgccaccgccacggggctcataactccttaagagcggttagtgtgtggtggctcgcactacaacctctctggatcatctacccccgtagcttgctcttttgtgcttgtgagcgacctcgtccttagccacgtcatattttgattttttgtttgttttgtttgtttgttgtatgcttttagtcatagctgattcgtactactcctgtttgcttcatggttcctgaatcccagagactccctgagcatgggtggctatcatgttggg

SEQ ID NO: 6 - protein, 561 aa, Rattus norvegicus
MGMPPLLFCWVSFVLPLFVAAGNCTDVYMHHEMISEGQPFPFNCTYPPVTNGAVNLTWHRTPSKSPISINRHVRIHQDQSWILFLPLALEDSGIYQCVIKDAHSCYRIAINLTVFRKHWCDSSNEESSINSSDEYQQWLPIGKSGSLTCHLYFPESCVLDSIKWYKGCEEIKVSKKFCPTGTKLLVNNIDVEDSGSYACSARLTHLGRIFTVRNYIAVNTKEVGSGGRIPNITYPKNNSIEVQLGSTLIVDCNITDTKENTNLRCWRVNNTLVDDYYNDFKRIQEGIETNLSLRNHILYTVNITFLEVKMEDYGHPFTCHAAVSAAYIILKRPAPDFRAYLIGGLMAFLLLAVSILYIYNTFKVDIVLWYRSTFHTAQAPDDEKLYDAYVLYPKYPRESQGHDVDTLVLKILPEVLEKQCGYKLFIFGRDEFPGQAVASVIDENIKLCRRLMVLVAPETSSFSFLKNLTEEQIAVYNALVQDGMKVILIELERVKDYSTMPESIQYIRQKHGAIQWDGDFTEQAQCAKTKFWKKVRYHMPPRRYPASPPVQLLGHTPRIPG

SEQ ID NO: 7 - protein, 573 aa, Artificial Sequence
  Humanized Il1r12
MGVTSLLFCGVFFLLLLFVAADGCKDIFMKNEILSASQPFAFNCTFPPITSGEVSVTWYKNSSKIPVSKIIQSRIHQDETWILFLPMEWGDSGVYQCVIKGRDSCHRIHVNLTVFEKHWCDTSIGGLPNLSDEYKQILHLGKDDSLTCHLHFPKSCVLGPIKWYKDCNEIKGERFTVLETRLLVSNVSAEDRGNYACQAILTHSGKQYEVLNGITVSITERAGYGGSVPKIIYPKNHSIEVQLGTTLIVDCNVTDTKDNTNLRCWRVNNTLVDDYYDESKRIREGVETHVSFREHNLYTVNITFLEVKMEDYGLPFMCHAGVSTAYIILQLPVPDFRAYLLGGLMAFLLLVVSVLFIYNSFKIDIMLWYRSAFHTAQAPDDEKLYDAYVLYPKYPRGSQGHDVDTLVLKILPEVLEKQCGYKLFIFGRDEFPGQAVASVIDENIKLCRRLMVFVAPESSSFGFLKNLSEEQIAVYNALIQHGMKVILIELEKVKDYSTMPESIQYIRQKHGAIQWDGDFTEQSQCAKTKFWKKVRYHMPPRRYPASSPVQLLGHIPCNCKAGKCNAATGLITP

SEQ ID NO: 8 - DNA, 888 bp, Homo sapiens
aaaacccaagtgcagtagaagccattgttcataatggtagggatacagggtccttcgtaacagattatcagtgtggcctatgctggaaagtctggtgacctctgattttttttgcttccaggtctttggccttggcactctttgtcatattagagttcctgggtctaggcctgggcaggattcataggtgcagctgcttctgctggaggtagactgcatccaacaaagtaagggtgctgggtgagttctgggagtatagattctgactggggtcactgctgggctggccgccagtctttcatctgacccagggttaaactgtggcttgggactgactcaggtcctctcttggggtcggtctgcacataaaaggactcctatccttggcagttctgaaacaacaccaccacaatggaaaaagcattgaaaattgacacacctcagcaggggagcattcaggatatcaatcatcgggtgtgggttcttcaggaccagacgctcatagcagtcccgaggaaggaccgtatgtctccagtcactattgccttaatctcatgccgacatgtggagacccttgagaaagacagagggaaccccatctacctgggcctgaatggactcaatctctgcctgatgtgtgctaaagtcggggaccagcccacactgcagctgaaggaaaaggatataatggatttgtacaaccaacccgagcctgtgaagtcctttctcttctaccacagccagagtggcaggaactccaccttcgagtctgtggctttccctggctggttcatcgctgtcagctctgaaggaggctgtcctctcatccttacccaagaactggggaaagccaacactactgactttgggttaactatgctgttttaa

SEQ ID NO: 9 - protein, 158 aa, Homo sapiens
MEKALKIDTPQQGSIQDINHRVWVLQDQTLIAVPRKDRMSPVTIALISCRHVETLEKDRGNPIYLGLNGLNLCLMCAKVGDQPTLQLKEKDIMDLYNQPEPVKSFLFYHSQSGRNSTFESVAFPGWFIAVSSEGGCPLILTQELGKANTTDFGLTMLF

SEQ ID NO: 10 - DNA, 883 bp, Mus musculus
taacctcctcttttcgtgttgtggataaaaggcttggaccttagtagagcttgtcagagaagctgagcacagtagtgggtgtagttctgtagtgtgcagacacattcctattcaatcagggtcaatctgcagattggcagctcagaaacaacatcaccataatgaataaggagaaagaactaagagcagcatcaccttcgcttagacatgttcaggatcttagtagtcgtgtgtggatcctgcagaacaatatcctcactgcagtcccaaggaaagagcaaacagttccagtcactattaccttgctcccatgccaatatctggacactcttgagacgaacaggggggatcccacgtacatgggagtgcaaaggccgatgagctgcctgttctgcacaaaggatggggagcagcctgtgctacagcttggggaagggaacataatggaaatgtacaacaaaaaggaacctgtaaaagcctctctcttctatcacaagaagagtggtacaacctctacatttgagtctgcagccttccctggttggttcatcgctgtctgctctaaagggagctgcccactcattctgacccaagaactgggggaaatcttcatcactgacttcgagatgattgtggtacattaaggtttttagacacattgctctgtggcactctctcaagatttcttggattctaacaagaagcaatcaaagacacccctaacaaaatggaagactgaaaagaaagctgagccctccctgggctgtttttccttggtggtgaatcagatgcagaacatcttaccatgttttcatccaaagcatttactgttggtttttacaaggagtgaattttttaaaataaaatcatttatctcatttgc

SEQ ID NO: 11 - protein, 160 aa, Mus musculus
MNKEKELRAASPSLRHVQDLSSRVWILQNNILTAVPRKEQTVPVTITLLPCQYLDTLETNRGDPTYMGVQRPMSCLFCTKDGEQPVLQLGEGNIMEMYNKKEPVKASLFYHKKSGTTSTFESAAFPGWFIAVCSKGSCPLILTQELGEIFITDFEMIVVH

SEQ ID NO: 12 - DNA, 869 bp, Rattus norvegicus
taatctcctcccttcatgttttggataaaaggcctggaccctagcagagcttgtcagagaagctgagcacagtagtggctgtagttctgtagtgtgcagatacattcctctgcaatcaggatcagtctgcagattggcagttcagaaacaacatcaccataatgaataaggataaagaactaagtgcagcaacaccttggtttagacatattcaggatcttagtagtcgtgtgtgggtccttcaagacaatattcttactgcagtcccaaggaaagagcaaacggttccagtcactatcaccttactcccatgccaatatctggacactcttgagaagaacaaaggggatcccatgtacctgggagtgaagaaacctcaaagttgtctgtcctgcacaaagaatggggagcagcctgtactacaacttcgggaagggaacatactggatatgtaccaccagaaggaacgtgtaaaagcctctctcttctatcacaagaagagtggtacaacctctacattcgagtctgcagccttccctggttggttcattgctgtctgctccaaagggagctgcccactcgttttgacccaagaacttgggaaaaccttcatcactgattttgagatgactgtagtacattaagattgctctgcagcactctctgaagatctctcggattctaacaagcaaccaaacacacccccaacaaaatacaagactgaaaagaaagctgagccctccctgggcttttttcccttggcaggtggatcagatgcagaacttcttaccatgttttcatccaaagcatttactgatggtttttacaagaagaaaacgtttttaattaaaatcatttatctcacttgc

SEQ ID NO: 13 - protein, 160 aa, Rattus norvegicus
MNKDKELSAATPWFRHIQDLSSRVWVLQDNILTAVPRKEQTVPVTITLLPCQYLDTLEKNKGDPMYLGVKKPQSCLSCTKNGEQPVLQLREGNILDMYHQKERVKASLFYHKKSGTTSTFESAAFPGWFIAVCSKGSCPLVLTQELGKTFITDFEMTVVH

SEQ ID NO: 14 - DNA, 1186 bp, Homo sapiens
cacgggttcctccccactctgtctttctcacctctccttcacttttcctagcctcctcaccaccatctgatctatcttgttctcttcacaaaaggctctgaagacatcatgaacccacaacgggaggcagcacccaaatcctatgctattcgtgattctcgacagatggtgtgggtcctgagtggaaattctttaatagcagctcctcttagccgcagcattaagcctgtcactcttcatttaatagcctgtagagacacagaattcagtgacaaggaaaagggtaatatggtttacctgggaatcaagggaaaagatctctgtctcttctgtgcagaaattcagggcaagcctactttgcagcttaagcttcagggctcccaagataacatagggaaggacacttgctggaaactagttggaattcacacatgcataaacctggatgtgagagagagctgcttcatgggaacccttgaccaatggggaataggagtgggtagaaagaagtggaagagttcctttcaacatcaccatctcaggaagaaggacaaagatttctcatccatgcggaccaacataggaatgccaggaaggatgtagaaataaggggaggaagattcccatctctacaatctttgagtgggtttgctatcaatgaaatgctacaaatggaataagttgcagaaatttttctcttttcttgggttctggagagtttgtaaaacaaggacactatgtatttttaaagagttggtaaatcttacctgtaaagctagagaaggtcggagtctttttaggagtagatttggactacataacctgtaaatgtgttttgtccagtccttagagtgttttttaaaaaattgtaaagtcaaggttttcatgaaaaatgggaagatcagacaacattgctcctgaattcccacagagcagcaagctactagagctcaatctgttatttcttttcctgatgtacaggggttaagtcctatggaagaaacagcagaattattcaaaattatttacataatgtgcaattattcactagagcatgaggagtgaaacgctctgtttagtatgtataacttaaaaggaacacatacaattaaaagtaattgaaagacatttcttcttaaaaattctataatcttacactggtaaaataaactagtttttcccatgt

SEQ ID NO: 15 - protein, 164 aa, Homo sapiens
MNPQREAAPKSYAIRDSRQMVWVLSGNSLIAAPLSRSIKPVTLHLIACRDTEFSDKEKGNMVYLGIKGKDLCLFCAEIQGKPTLQLKLQGSQDNIGKDTCWKLVGIHTCINLDVRESCFMGTLDQWGIGVGRKKWKSSFQHHHLRKKDKDFSSMRTNIGMPGRM

SEQ ID NO: 16 - DNA, 790 bp, Mus musculus
gactggcctcattgcctgctgtcataacttcgatcccagagacaagacttctttggaccaaggcaatgatggctttccctccacaatcttgtgtacatgttcttcctccaaagagtattcaaatgtgggaaccgaatcataacactatgcatggatcctcacaatctcccagaaactacagggttcatgactcacaacagatggtatgggtcctgactggaaatactttaacagcagttcctgctagcaacaatgtcaagcctgtcattcttagcttgatagcatgtagagacacggaattccaagatgtaaagaaaggtaatctagttttcctgggaatcaagaacagaaatctctgcttctgctgtgttgagatggagggcaaaccaactttgcagcttaaggaagtagacatcatgaatttgtacaaagagagaaaagcacaaaaagcctttctgttctatcatggcatagagggctccacttctgtctttcagtcagtcctctatcctggctggtttatagccacctcttccatagaaagacagacaatcatcctcacacatcagcggggtaaattggttaacactaacttctacatagagtctgagaagtaaatccaacatgggtcatatgtggccagctccaggccacagaatcaaactgttgaagaatcttctacttgaaaacatagcaagcctcttagaagaccaccatgccatgtcttcaccagacatccatgtctaaaatgccactcatttgaatatcattccagcatgaagcccatgaa

SEQ ID NO: 17 - protein, 183 aa, Mus musculus
MMAFPPQSCVHVLPPKSIQMWEPNHNTMHGSSQSPRNYRVHDSQQMVWVLTGNTLTAVPASNNVKPVILSLIACRDTEFQDVKKGNLVFLGIKNRNLCFCCVEMEGKPTLQLKEVDIMNLYKERKAQKAFLFYHGIEGSTSVFQSVLYPGWFIATSSIERQTIILTHQRGKLVNTNFYIESEK

SEQ ID NO: 18 - DNA, 587 bp, Rattus norvegicus
ggcgtgggtcctggctggaaattctttgacagcggttcctgctagcaacagcgtcaaatctgtcattcttagcttgatagcatgtagagacatggaattccaagatgaaaagaagggtaatctagttttcctgggaatcaaaggcagaagtctctgcctcttctgtgctgagatcgagggcaaaccgactttgcagcttaaggatgtagacatcatggatttgtacaatgagaaaaaagcacagaaagcctttctcttctaccatggcatagagggatctacttctgtctttcagtcagtcttgtatcctggctggtttatagccacctcttccacagcaagacaaacaatcattcttacacaggagaggggtgaagctaataacactaacttctacttagagtctgagaattagatctaccatgggccatatgtggccagttgcaggccaaagaatcaaactgttggagaatcttttacttgaaaacatagcaagacatcttagaagaccaccatgtttcctcttctcctgacatccatgtctgaaatgccattcattggtataagagaataaaaaatagggctgg

SEQ ID NO: 19 - protein, 179 aa, Rattus norvegicus
MMAFPPQSHVCFTPPKSSDFDNINKGVQAFPSTYRVHDSQHKAWVLAGNSLTAVPASNSVKSVILSLIACRDMEFQDEKKGNLVFLGIKGRSLCLFCAEIEGKPTLQLKDVDIMDLYNEKKAQKAFLFYHGIEGSTSVFQSVLYPGWFIATSSTARQTIILTQERGEANNTNFYLESEN

SEQ ID NO: 20 - DNA, 1212 bp, Homo sapiens
gaagctgctggagccacgattcagtcccctggactgtagataaagaccctttcttgccaggtgctgagacaaccacactatgagaggcactccaggagacgctgatggtggaggaagggccgtctatcaatcaatgtgtaaacctattactgggactattaatgatttgaatcagcaagtgtggacccttcagggtcagaaccttgtggcagttccacgaagtgacagtgtgaccccagtcactgttgctgttatcacatgcaagtatccagaggctcttgagcaaggcagaggggatcccatttatttgggaatccagaatccagaaatgtgtttgtattgtgagaaggttggagaacagcccacattgcagctaaaagagcagaagatcatggatctgtatggccaacccgagcccgtgaaacccttccttttctaccgtgccaagactggtaggacctccacccttgagtctgtggccttcccggactggttcattgcctcctccaagagagaccagcccatcattctgacttcagaacttgggaagtcatacaacactgcctttgaattaaatataaatgactgaactcagcctagaggtggcagcttggtctttgtcttaaagtttctggttcccaatgtgttttcgtctacattttcttagtgtcattttcacgctggtgctgagacaggggcaaggctgctgttatcatctcattttataatgaagaagaagcaattacttcatagcaactgaagaacaggatgtggcctcagaagcaggagagctgggtggtataaggctgtcctctcaagctggtgctgtgtaggccacaaggcatctgcatgagtgactttaagactcaaagaccaaacactgagctttcttctaggggtgggtatgaagatgcttcagagctcatgcgcgttacccacgatggcatgactagcacagagctgatctctgtttctgttttgctttattccctcttgggatgatatcatccagtctttatatgttgccaatatacctcattgtgtgtaatagaaccttcttagcattaagaccttgtaaacaaaaataattcttgtgttaagttaaatcatttttgtcctaattgtaatgtgtaatcttaaagttaaataaactttgtgtatttatataataataaagctaaaactgatataaaataaagaaagagtaaactg

SEQ ID NO: 21 - protein, 169 aa, Homo sapiens
MRGTPGDADGGGRAVYQSMCKPITGTINDLNQQVWTLQGQNLVAVPRSDSVTPVTVAVITCKYPEALEQGRGDPIYLGIQNPEMCLYCEKVGEQPTLQLKEQKIMDLYGQPEPVKPFLFYRAKTGRTSTLESVAFPDWFIASSKRDQPIILTSELGKSYNTAFELNIND

SEQ ID NO: 22 - DNA, 1647 bp, Mus musculus
atcattacacctgggagctgcccaagctgggatttggtcttctagactttccataaggactctttcttgccatgtacctacaaacctacaaaaccctttgagtgcgcctctgagtgtggagctttctgcagttcagggttcagtgaatggacagatctgtcttgctgtaagtgatcctgtgagcgatcctgtgagcgatcctgtgagcgatcctgtgagcgatcctgtgagcgatcctgtgagtgatcctgtgagcaatcctgtgagagctctgtgcaccagaacaagatcacgatggaaaacaatgaaaaaaaaaacattgtgtatggaagtgatgttgagatggaacacgagagagctgggctatttgtatcttcagctatgttttctaaacacccattttctacacacatctcaggaagagaaactcctgactttggggaggtttttgacttggaccagcaggtgtggatctttcgtaatcaggcccttgtgacagttccacgaagccacagagtaaccccagtcagcgtgactatcctcccatgcaagtacccagagtctcttgaacaggacaaagggattgccatttatttgggaattcagaatccagataaatgcctgttttgtaaggaagttaatggacaccctactttgctgctaaaggaagagaagattttggatttgtaccaccaccctgagccaatgaagccattcctgttttaccacacccggacaggtggaacatccacctttgaatcagtggctttccctggccactatattgcctcctccaagactggcaaccccatcttcctcacatcaaaaaagggagaatattacaacattaacttcaatttagatataaagtcttaaactcagcatggaagtggagggttggttagaactcttcctcttaaaacatcaaacctctaatatgttatcatttgtttgatctatggtattttcatactgaaaggtaagcaggaccaacattatctcctttcatagatgaagaagcaacaaaataatgcatactccaaagtcggtgggattggagtggtgtaaggatgttctctaagactgaagtggtccaatctataagacatcatgtctgagaaatagggtgctgtgccacagtgtataaaacctagaatgccctgtgtgtgagtggtgacatcctcatttccagccattggcctgattcataccatgttttcacacatttgtaatatcaactccttgcatttggatagcagaggcctcacaatgacatttgcctcaacagctaatagctttgatctttcaatgctgtgtagatctgaatacactagaaaaggaattagaatcctgagtgaatgaactgtgaggagccgccctcacatttgccattataagatggcactgacagctgtgttctaagtggtaaacatagtctgcacacatgcaggggcagttttcccaccatgtgttctgcctttcccgtgatgacaactgggccgatgggctgcagccaatcagggagtaatacgtcctaggtggaggataattctccttaaaagggacggggttctggcactctctcccttccttgcttgctctcttgcactctggctcctgaagatgtaagcaataaagctttgccgc

SEQ ID NO: 23 - protein, 164 aa, Mus musculus
MFSKHPFSTHISGRETPDFGEVFDLDQQVWIFRNQALVTVPRSHRVTPVSVTILPCKYPESLEQDKGIAIYLGIQNPDKCLFCKEVNGHPTLLLKEEKILDLYHHPEPMKPFLFYHTRTGGTSTFESVAFPGHYIASSKTGNPIFLTSKKGEYYNINFNLDIKS

SEQ ID NO: 24 - DNA, 1395 bp, Rattus norvegicus
ggaagctgcccaagctgggatttgatcttctgaactttccataaggactctttcttgccaggcaccagaacaagctcatgatggaaaacaatgaaaaaaatcgttacatatgggtgtgatgttgagatgtgacactaacgaactgggctatttgtatcttcagctatgtcctctaaatacccacattctccatgtactgcctcagcaggaaaagaaactcctgaccttgggcaggtttctgatgtggatcagcaggtgtggatctttcgtgatcaggcccttgtgacagttccacgaagccacactgtaactccagtcactgtgactgtcctcccatgcaagtacccagagtctcttgagcagggcaaagggactcccatttatttgggaattcaaaatccagataaatgcctgttttgtaaggaagttaatggacaccccactttgctcctgaaggaagagaagattttgaatttgtaccaccatcctgagccaatgaagccattcctgttttaccacaccctgacaggtgcaacgtccacctttgaatcagtggttttccctggcagctttattgcctcctccaagattggcaaacccatcttcctcacatcaaaaaagggagaacattacaacattcacttcagtttagatataatttagatataaagtcttgaactcagaatggaggtggagggttggttagaactcttataacttcaaacctctaatatgctatcatttgtttgatgtgtggttgtttcatactgagaagtgagcaaaaccaacattatctcatttcatagatgaagaagcaacaaaacagaatgtgtactccaaagtaggttggatgggagtggtgtaaggctctcctctaagactgaagtggtccaacccataaggcatcatgcctttctcaggtgctattatagggtgctgtgccacagtatataaaaactagaatgccccatgtgtgagtagcaacatcctcacttccagtcattggcctgattcataccaggttttcacacacttgtaataccaattccttgcatttggatagcaggagcctcacaatgacatttgctgccaacagctgatagctttgatccttcagcaactgactgctacgtggatctgaagacgccagaaaaggaattagaatcctaagtgaacgaacagtttttaaaatgtctagaactatttaaactatgttagaatacagtggtttatccttgaaaggtaaggatactgcctggtaaatcaaaaacagttaggtcaataaactcagcttgaacaattctttcctggaaacaatgtgtacaagtaatgattaaaacattaccttttattattctagacttccataaaaaaaaaaaaaaaaaaaaaaaaaaa

SEQ ID NO: 25 - protein, 165 aa, Rattus norvegicus
MSSKYPHSPCTASAGKETPDLGQVSDVDQQVWIFRDQALVTVPRSHTVTPVTVTVLPCKYPESLEQGKGTPIYLGIQNPDKCLFCKEVNGHPTLLLKEEKILNLYHHPEPMKPFLFYHTLTGATSTFESVVFPGSFIASSKIGKPIFLTSKKGEHYNIHFSLDII

SEQ ID NO: 26 - DNA, 108 bp, Artificial Sequence
  Synthetic Oligonucleotide
tacatttgaaggtcttagcattatgcttctaaatgactgggctagtttgggcgatcgcgacaagaagggttgatttactctgtaggtgagtacagagtaaagaactct

SEQ ID NO: 27 - DNA, 140 bp, Artificial Sequence
  Synthetic Oligonucleotide
caccctgagcacatggggaatccttcttgggttgcaacatgtggaaggacctcgagataacttcgtataatgtatgctatacgaagttatatgcatggcctccgcgccgggttttggcgcctcccgcgggcgcccccctc

SEQ ID NO: 28 - DNA, 181 bp, Artificial Sequence
  Synthetic Oligonucleotide
tttcactgcattctagttgtggtttgtccaaactcatcaatgtatcttatcatgtctggaataacttcgtataatgtatgctatacgaagttatgctagtaactataacggtcctaaggtagcgagctagccagaatcaatgacaaagatgaagaatatatttaacctcataaacttggtt

SEQ ID NO: 29 - DNA, 177 bp, Artificial Sequence
  Synthetic Oligonucleotide
caccctgagcacatggggaatccttcttgggttgcaacatgtggaaggacctcgagataacttcgtataatgtatgctatacgaagttatgctagtaactataacggtcctaaggtagcgagctagccagaatcaatgacaaagatgaagaatatatttaacctcataaacttggtt

SEQ ID NO: 30 - DNA, 100 bp, Artificial Sequence
  Synthetic Oligonucleotide
ctggctctgtcaactagattggaaggcatgcggagctgccagtctcaactcgtcgacgtcactctcctttcccactgcatgtgaagcatttgagtgtctg

SEQ ID NO: 31 - DNA, 140 bp, Artificial Sequence
  Synthetic Oligonucleotide
tgcactcagaaaagacaagtattcacattttttcttgtggctgatctggactcgagataacttcgtataatgtatgctatacgaagttatatgcatggcctccgcgccgggttttggcgcctcccgcgggcgcccccctc

SEQ ID NO: 32 - DNA, 181 bp, Artificial Sequence
  Synthetic Oligonucleotide
tttcactgcattctagttgtggtttgtccaaactcatcaatgtatcttatcatgtctggaataacttcgtataatgtatgctatacgaagttatgctagtaactataacggtcctaaggtagcgagctagcctatgcctgcacagcccttccataggtactaaggatttaaactctcgttt

SEQ ID NO: 33 - DNA, 177 bp, Artificial Sequence
  Synthetic Oligonucleotide
tgcactcagaaaagacaagtattcacattttttcttgtggctgatctggagtcgagataacttcgtataatgtatgctatacgaagttatgctagtaactataacggtcctaaggtagcgagctagcctatgcctgcacagcccttccataggtactaaggatttaaactctcgttt

SEQ ID NO: 34 - DNA, 24 bp, Artificial Sequence
  Synthetic Oligonucleotide
gggtccattatttgagactttcca

SEQ ID NO: 35 - DNA, 25 bp, Artificial Sequence
  Synthetic Oligonucleotide
agctttctgctggccccattacttg

SEQ ID NO: 36 - DNA, 19 bp, Artificial Sequence
  Synthetic Oligonucleotide
gcatgtgcctgtcttcaca

SEQ ID NO: 37 - DNA, 25 bp, Artificial Sequence
  Synthetic Oligonucleotide
gagtggtacaacctctacatttgag

SEQ ID NO: 38 - DNA, 23 bp, Artificial Sequence
  Synthetic Oligonucleotide
ctgcagccttccctggttggttc

SEQ ID NO: 39 - DNA, 20 bp, Artificial Sequence
  Synthetic Oligonucleotide
agtgggcagctccctttaga

SEQ ID NO: 40 - DNA, 19 bp, Artificial Sequence
  Synthetic Oligonucleotide
cccactgcatgtgaagcat

SEQ ID NO: 41 - DNA, 22 bp, Artificial Sequence
  Synthetic Oligonucleotide
ttgagtgtctgcacctgagcca

SEQ ID NO: 42 - DNA, 23 bp, Artificial Sequence
  Synthetic Oligonucleotide
ggagacctcttattagcctgtga

SEQ ID NO: 43 - DNA, 20 bp, Artificial Sequence
  Synthetic Oligonucleotide
cacctgccctaagtcatctc

SEQ ID NO: 44 - DNA, 22 bp, Artificial Sequence
  Synthetic Oligonucleotide
tacagcaagagcagaggccaca

SEQ ID NO: 45 - DNA, 21 bp, Artificial Sequence
  Synthetic Oligonucleotide
gcctgcagagaagcaatgttc

SEQ ID NO: 46 - DNA, 19 bp, Artificial Sequence
  Synthetic Oligonucleotide
cagccgctacacaccacaa

SEQ ID NO: 47 - DNA, 24 bp, Artificial Sequence
  Synthetic Oligonucleotide
ccagctgctacacaaatgcagggc

SEQ ID NO: 48 - DNA, 20 bp, Artificial Sequence
  Synthetic Oligonucleotide
cgtcatctcctgccagttca

SEQ ID NO: 49 - DNA, 21 bp, Artificial Sequence
  Synthetic Oligonucleotide
ctgctgctcagagcattgaaa

SEQ ID NO: 50 - DNA, 23 bp, Artificial Sequence
  Synthetic Oligonucleotide
ccatggccagggaaggcttacta

SEQ ID NO: 51 - DNA, 22 bp, Artificial Sequence
  Synthetic Oligonucleotide
cgcctccgactgaacatatgac

SEQ ID NO: 52 - DNA, 25 bp, Artificial Sequence
  Synthetic Oligonucleotide
cctgatatgcatctttccctatgga

SEQ ID NO: 53 - DNA, 23 bp, Artificial Sequence
  Synthetic Oligonucleotide
atggcacctcagaccagacccac

SEQ ID NO: 54 - DNA, 24 bp, Artificial Sequence
  Synthetic Oligonucleotide
ggcagcaataatactgggacaaac

SEQ ID NO: 55 - DNA, 21 bp, Artificial Sequence
  Synthetic Oligonucleotide
ggccaggaaacacatctgaag

SEQ ID NO: 56 - DNA, 27 bp, Artificial Sequence
  Synthetic Oligonucleotide
agcagtgactctaaatgctcagtgtga

SEQ ID NO: 57 - DNA, 23 bp, Artificial Sequence
  Synthetic Oligonucleotide
gcctcactccaacaacattatga